European Patent Specification EP 3 978 598 B1, published August 28, 2024. Title: HUMAN-DERIVED BACTERIA THAT INDUCE PROLIFERATION OR ACCUMULATION OF REGULATORY T CELLS. Applicant: UNIVERSITY OF TOKYO SCHOOL CORPORATION, AZABU VETERINARY MEDICINE EDUCATIONAL INSTITUTION HONDA, Kenya ATARASHI, Koji TANOUE, Takeshi HATTORI, Masahira MORITA, Hidetoshi. Application Not Yet Assigned. The sequence listing filed with the application follows.

SEQUENCE LISTING (123 sequences)

SEQ ID NO: 1 - DNA, 23 bp, Artificial Sequence
  Primer, Foxp3
ggcaatagttccttcccagagtt

SEQ ID NO: 2 - DNA, 22 bp, Artificial Sequence
  Primer, Foxp3
gggtcgcatattgtggtacttg

SEQ ID NO: 3 - DNA, 23 bp, Artificial Sequence
  Primer, CTLA4
ccttttgtagccctgctcactct

SEQ ID NO: 4 - DNA, 21 bp, Artificial Sequence
  Primer, CTLA4
gggtcacctgtatggcttcag

SEQ ID NO: 5 - DNA, 21 bp, Artificial Sequence
  Primer, GITR
tcagtgcaagatctgcaagca

SEQ ID NO: 6 - DNA, 19 bp, Artificial Sequence
  Primer, GITR
acaccggaagccaaacaca

SEQ ID NO: 7 - DNA, 27 bp, Artificial Sequence
  Primer, IL-10
gattttaataagctccaagaccaaggt

SEQ ID NO: 8 - DNA, 27 bp, Artificial Sequence
  Primer, IL-10
cttctatgcagttgatgaagatgtcaa

SEQ ID NO: 9 - DNA, 21 bp, Artificial Sequence
  Primer, GAPDH
cctcgtcccgtagacaaaatg

SEQ ID NO: 10 - DNA, 20 bp, Artificial Sequence
  Primer, GAPDH
tctccactttgccactgcaa

SEQ ID NO: 11 - DNA, 20 bp, Artificial Sequence
  Primer, Mmp2
ggacattgtctttgatggca

SEQ ID NO: 12 - DNA, 20 bp, Artificial Sequence
  Primer, Mmp2
cttgtcacgtggtgtcactg

SEQ ID NO: 13 - DNA, 20 bp, Artificial Sequence
  Primer, Mmp9
tctctggacgtcaaatgtgg

SEQ ID NO: 14 - DNA, 19 bp, Artificial Sequence
  Primer, Mmp9
gctgaacagcagagccttc

SEQ ID NO: 15 - DNA, 20 bp, Artificial Sequence
  Primer, Mmp13
aggtctggatcactccaagg

SEQ ID NO: 16 - DNA, 19 bp, Artificial Sequence
  Primer, Mmp13
tcgcctggaccataaagaa

SEQ ID NO: 17 - DNA, 20 bp, Artificial Sequence
  Primer, Ido1
agaggatgcgtgactttgtg

SEQ ID NO: 18 - DNA, 20 bp, Artificial Sequence
  Primer, Ido1
atacagcagaccttctggca

SEQ ID NO: 19 - DNA, 302 bp, Artificial Sequence
  OTU136
gatgaacgctggcggcgtgcctaatacatgcaagtcgaacgcgagcacttgtgctcgagtggcgaacgggtgagtaatacataagtaacctgccctttacagggggataactattggaaacgatagctaagaccgcataggtaaagataccgcatggtaagtttattaaaagtgccaaggcactggtagaggatggacttatggcgcattagctagttggtgaggtaacggctcaccaaggcgacgatgcgtagccgacctgagagggtgaccggccacactgggactgagacacggcccag

SEQ ID NO: 20 - DNA, 303 bp, Artificial Sequence
  OTU46
gatgaacgctggcggcgtgcctaatacatgcaagtcgaacgcgagcacttgtgctcgagtggcgaacgggtgagtaatacataagtaacctgccctagacagggggataactattggaaacgatagctaagaccgcataggtacggacactgcatggtgaccgtattaaagtgcctcaaagcactggtagaggatggacttatggcgcattagctggttggcggggtaacggcccaccaaggcgacgatgcgtagccgacctgagagggtgaccggccacactgggactgagacacggcccag

SEQ ID NO: 21 - DNA, 324 bp, Artificial Sequence
  OTU221
gatgaacgctggcggcgtgcttaacacatgcaagtcgaacggggtgctcatgacggaggattcgtccaacggattgagttacccagtggcggacgggtgagtaacgcgtgaggaacctgccttggagaggggaataacactccgaaaggagtgctaataccgcatgatgcagttgggtcgcatggctctgactgccaaagatttatcgctctgagatggcctcgcgtctgattagctagtaggcggggtaacggcccacctaggcgacgatcagtagccggactgagaggttgaccggccacattgggactgagacacggccca

SEQ ID NO: 22 - DNA, 325 bp, Artificial Sequence
  OTU9
gatgaacgctggcggcggtgcttaacacatgcaagtcgagcgaagcggtttcgagtgaagttttggatggaattgaaattgacttagcggcggacgggtgagtaacgcgtgggtaacctgccttacactgggggataacagttagaaatgactgctaataccgcataagcgcacagggccgcatggtctggtgcgaaaaactccggtggtgtaagatggacccgcgtctgattaggtagttggtggggtaacggcccaccaagccgacgatcagtagccgacctgagagggtgaccggccacattgggactgagacacggcccaa

SEQ ID NO: 23 - DNA, 325 bp, Artificial Sequence
  OTU296
gatgaacgctggcggcgtgcctaacacatgcaagtcgaacgaagcgcctggccccgacttcttcggaacgaggagccttgcgactgagtggcggacgggtgagtaacgcgtgggcaacctgccttgcactgggggataacagccagaaatggctgctaataccgcataagaccgaagcgccgcatggcgcagcggccaaagccccggcggtgcaagatgggcccgcgtctgattaggtagttggcggggtaacggcccaccaagccgacgatcagtagccgacctgagagggtgaccggccacattgggactgagacacggccca

SEQ ID NO: 24 - DNA, 323 bp, Artificial Sequence
  OTU21
gatgaacgctggcggcgtgcttaacacatgcaagtcgagcgaagcgctaagacagatttcttcggattgaagtctttgtggctgagcggcggacgggtgagtaacgcgtgggtaacctgcctcatacagggggataacagttagaaatgactgctaataccgcataagcgcacaggaccgcatggtctggtgtgaaaaactccggtggtatgagatggacccgcgtctgattagctagttggaggggtaacggcccaccaaggcgacgatcagtagccggcctgagagggtgaacggccacattgggactgagacacggccca

SEQ ID NO: 25 - DNA, 322 bp, Artificial Sequence
  OTU166
gatgaacgctggcggcgtgcctaacacatgcaagtcgaacgaagcaattaaaatgaagtttcggatggattttgattgactgagtggcggacgggtgagtaacgcgtggataacctgcctcacactgggggataacagttagaaatgactgctaataccgcataagcgcacagtaccgcatggtacggtgtgaaaaactccggtggtgtgagatggatccgcgtctgattagccagttggcggggtaacggcccaccaaagcgacgatcagtagccgacctgagagggtgaccggccacgattgggactgagacacggccca

SEQ ID NO: 26 - DNA, 313 bp, Artificial Sequence
  OTU73
gatgaacgctggcggcatgcctaatacatgcaagtcgaacgaagtgaagatagcttgctatcggagcttagtggcgaacgggtgagtaacacgtagataacctgcctgtatgaccgggataacagttggaaacgactgctaataccggataggcagagaggaggcatctcttctctgttaaagttgggatacaacgcaaacagatggatctgcggtgcattagctagttggtgaggtaacggcccaccaaggcgatgatgcatagccggcctgagagggcgaacggccacattgggactgagacacggcccaa

SEQ ID NO: 27 - DNA, 325 bp, Artificial Sequence
  OTU174
gatgaacgctggcggcgtgcttaacacatgcaagtcgaacgaagcattttggaaggaagttttcggatggaattccttaatgactgagtggcggacgggtgagtaacgcgtggggaacctgccctatacagggggataacagctggaaacggctgctaataccgcataagcgcacagaatcgcatgattcggtgtgaaaagctccggcagtataggatggtcccgcgtctgattagctggttggcggggtaacggcccaccaaggcgacgatcagtagccggcttgagagagtggacggccacattgggactgagacacggccca

SEQ ID NO: 28 - DNA, 323 bp, Artificial Sequence
  OTU14
gatgaacgctggcggcgtgcttaacacatgcaagtcgagcgaagcggtttcaatgaagttttcggatggaattgaaattgacttagcggcggacgggtgagtaacgcgtgggtaacctgccttacactgggggataacagttagaaatgactgctaataccgcataagcgcacagggccgcatggtctggtgtgaaaaactccggtggtgtaagatggacccgcgtctgattaggtagttggtggggtaacggccaccaagccgacgatcagtagccgacctgagagggtgaccggccacattggggactgagacacggccca

SEQ ID NO: 29 - DNA, 323 bp, Artificial Sequence
  OTU55
gatgaacgctggcggcgtgcctaacacatgcaagtcgaacgaagttacacggaggaagttttcggatggaatcggtataacttagtggcggacgggtgagtaacgcgtgggaaacctgccctgtaccgggggataacacttagaaataggtgctaataccgcataagcgcacggaaccgcatggttccgtgtgaaaaactaccggtggtacaggatggtcccgcgtctgattagccagttggcagggtaacggcctaccaaagcgacgatcagtagccggcctgagagggtgaacggccacattgggactgagacacagccca

SEQ ID NO: 30 - DNA, 325 bp, Artificial Sequence
  OTU337
gacgaacgctggcggcgcgcctaacacatgcaagtcgaacggagcttacgttttgaagttttcggatggatgaatgtaagcttagtggcggacgggtgagtaacacgtgagcaacctgcctttcagagggggataacagccggaaacggctgctaataccgcatgatgttgcgggggcacatgcccctgcaaccaaaggagcaatccgctgaaagatgggctcgcgtccgattagccagttggcggggtaacggcccaccaaagcgacgatcggtagccggactgagaggttgaacggccacattgggactgagacacggcccag

SEQ ID NO: 31 - DNA, 324 bp, Artificial Sequence
  OTU314
gatgaacgctggcggcgtgcctaacacatgcaagtcgagcgaagcgctgttttcagaatcttcggaggaagaggacagtgactgagcggcggacgggtgagtaacgcgtgggcaacctgcctcatacagggggataacagttagaaatgactgctaataccgcataagcgcacaggaccgcatggtgtagtgtgaaaaactccggtggtatgagatggacccgcgtctgattaggtagttggtggggtaaggccgtaccaagccgacgatcagtagccgacctgagagggtgaccggccacattggggactgagacacggccca

SEQ ID NO: 32 - DNA, 325 bp, Artificial Sequence
  OTU195
gatgaacgctggcggcgtgcctaacacatgcaagtcgaacgaagcattttagatgaagttttcggatggattctgagatgactgagtggcggacgggtgagtaacacgtggataacctgcctcacactgggggacgaacagttagaaatgactgctaataccgcataagcgcacagtaccgcatggtacggtgtgaaaaactccggtggtgtgagatggatccgcgtctgattagccagttggcgggtaacggcccaccgaaagcgacgatcagtagccgacctgagagggtgaccggccacattgggactgagacacggcccaa

SEQ ID NO: 33 - DNA, 324 bp, Artificial Sequence
  OTU306
gatgaacgctggcggcgtgcctaacacatgcaagtcgaacgaagcgacttaacggaagttttcggatggaagttgaattgactgagtggcggacgggtgagtaacgcgtgggtaacctgccttgtactgggggacgaacagttagaaatgactgctaataccgcataagcgcacagtatcgcatgatacagtgtgaaaaactccggtggtacaagatggacccgcgtctgattagctagttggtaaggtaacggcttaccaaggcgacgatcagtagccgacctgagagggtgaccggccacattgggactgagacacggccca

SEQ ID NO: 34 - DNA, 324 bp, Artificial Sequence
  OTU87
gatgaacgctggcggcgtgcttaacacatgcaagtcgagcgaagcgctttacttagatttcttcggattgaaagttttgcgactgagcggcggacgggtgagtaacgcgtgggtaacctgcctcatacagggggataacagttagaaatgactgctaataccgcataagaccacagtaccgcatggtacagtgggaaaaactccggtggtatgagatggacccgcgtctgattagctagttggtaaggtaacggcttaccaaggcgacgatcagtagccgacctgagagggtgaccggccacattgggactgagacacggccca

SEQ ID NO: 35 - DNA, 325 bp, Artificial Sequence
  OTU86
  misc_feature (49)..(49): n is a, c, g, or t
gatgaacgctggcggcgtgcttaacacatgcaagtcgaacgaagcattnttggaaggaagtttcggatggaattccttaatgactgagtggcggacgggtgagtaacgcgtggggaacctaccctatacagggggataacagctggaaacggctgctaataccgcataagcgcacagaatcgcatgattcggtgtgaaaagctccggcagtataggatggtcccgcgtctgattagctggttggcgggtaacggcccaccaaggcgacgatcagtagccggcttgagagagtggacggccacattgggactgagacacggcccaa

SEQ ID NO: 36 - DNA, 323 bp, Artificial Sequence
  OTU152
gatgaacgctggcggcgtgcctaacacatgcaagtcgaacgaagttagacagaggaagttttcggatggaatcggtataacttagtggcggacgggtgagtaacgcgtgggaaacctgccctgtaccgggggataacacttagaaataggtgctaataccgcataagcgcacggaaccgcatgggttctgtgtgaaaactccggtggtacaggatggtcccgcgtctgattagccagttggcagggtaacggcctaccaaagcgacgatcagtagccggcctgagagggtgaacggccacattgggactgagacacggcccaa

SEQ ID NO: 37 - DNA, 326 bp, Artificial Sequence
  OTU253
gacgaacgctggcggcgtgcttaacacatgcaaatcgaacggagcacccttgactgaggtttcggccaaatgataggaatgcttagtggcggactggtgagtaacgcgtgaggaacctgccttccagagggggacaacagttggaaacgactgctaataccgcatgacgcatgaccggggcatcccgggcatgtcaaagattttatcgctggaagatggcctcgcgtctgattagctagatggtggggtaacggcccaccatggcgacgatcagtagccggactgagaggttgaccggccacattgggactgagatacgggcccag

SEQ ID NO: 38 - DNA, 326 bp, Artificial Sequence
  OTU259
gatgaacgctggcggcgtgcttaacacatgcaagtcgagcgaagcgctttacttagatttcttcggattgaaaagttttgcgactgagcggcggacgggtgagtaacgcgtgggtaacctgcctcatacagggggataacagttagaaatgactgctaataccgcataagaccacggtaccgcatggtacagtgggaaaaactccggtggtatgagatggacccgcgtctgattagctagttggtaaggtaacggcttaccaaggcgacgatcagtagccgacctgagagggtgaccggcacattgggacctgagacacggcccaa

SEQ ID NO: 39 - DNA, 327 bp, Artificial Sequence
  OTU281
gatgaacgctggcggcgtgcctaacacatgcaagtcgaacgaagcgcttccgcctgattttcttcggagatgaaggcggctgcgactgagtggcggacgggtgagtaacgcgtgggcaacctgccttgcactgggggataacagccagaaatggctgctaataccgcataagaccgaagcgccgcatggcgctgcggccaaagccccggcggtgcaagatgggcccgcgtctgattaggtagttggcggggtaacggcccaccaagccgacgatcagtagccgacctgagagggtgaccggccacattgggactgagacacggccca

SEQ ID NO: 40 - DNA, 322 bp, Artificial Sequence
  OTU288
gatgaacgctggcggcgtgcctaacacatgcaagtcgaacggagttatgcagaggaagttttcggatggaatcggcgtaacttagtggcggacgggtgagtaacgcgtgggaaacctgccctgtaccgggggataacacttagaaataggtgctaataccgcataagcgcacagcttcacatgaagcagtgtgaaaaactccggtggtacaggatggtcccgcgtctgattagccagttggcagggtaacggcctaccaaagcgacgatcagtagccggcctgagagggtgaacggccacattgggactgagacacggccca

SEQ ID NO: 41 - DNA, 324 bp, Artificial Sequence
  OTU334
gatgaacgctggcggcgtgcctaacacatgcaagtcgaacgaagcatcccataggaagttttcggatggaatatgggatgactgagtggcggacgggtgagtaacgcgtggataacctgcctcacactgggggataacagttagaaatggctgctaataccgcataagcgcacagtaccgcatggtacggtgtgaaaaacccaggtggtgtgagatggatccgcgtctgattagccagttggcggggtaacggcccaccaaagcgacgatcagtagccgacctgagagggtgaccggccacattggggactgagacacggccca

SEQ ID NO: 42 - DNA, 324 bp, Artificial Sequence
  OTU359
gatgaacgctggcggcgtgcctaacacatgcaagtcgaacgaagttatatcgaggaagttttcggatggaatcagtataacttagtggcggacgggtgagtaacgcgtgggaaacctgccctgtaccgggggataacacttagaaataggtgctaataccgcataagcgcacagcttcacatgaaagcagtgtgaaaaactccggtggtacaggatggtcccgcgtctgattagccagttggcagggtaacggcctaccaaagcgacgatcagtagccggcctggagagggtgaacggccacattgggactgagacacggcccg

SEQ ID NO: 43 - DNA, 321 bp, Artificial Sequence
  OTU362
gatgaacgctggcggcgtgcttaacacatgcaagtcgagcgaagcggtttcgatgaagttttcggatggatttgaaatcgacttagcggcggacgggtgagtaacgcgtgggtaacctgccttacactggggataacagttagaaatgactgctaataccgcataagcgcacagggccgcatggtccggtgtgaaaactccggtggtgtaagatggacccgcgtctgattaggtagttggtgggtaacggcccaccaagccgacgatcagtagccgacctgagagggtgaccggccacattgggactgagacacggcccaa

SEQ ID NO: 44 - DNA, 323 bp, Artificial Sequence
  OTU367
gatgaacgctggcggcgtgcctaacacatgcaagtcgaacgaagttacacagaggaagttttcggatggaatcggtataacttagtggcggacgggtgagtaacgcgtgggaaacccgccctgtaccgggggataacacttagaaataggtgctaataccgcataagcgcacagcttcacatgaagcagtgtgaaaactccggtaggtacaggatggtcccgcgtctgattagccagttggcagggtaacggcctaccaaagcgacgatcagtagccggcctgagagggtcaacggccacattgggactgagacacggcccaa

SEQ ID NO: 45 - DNA, 17 bp, Artificial Sequence
  Primer, total bacteria
ggtgaatacgttcccgg

SEQ ID NO: 46 - DNA, 22 bp, Artificial Sequence
  Primer, total bacteria
tacggctaccttgttacgactt

SEQ ID NO: 47 - DNA, 20 bp, Artificial Sequence
  Primer, Clostridium cluster XIVa (Clostridium coccoides subgroup)
aaatgacggtacctgactaa

SEQ ID NO: 48 - DNA, 22 bp, Artificial Sequence
  Primer, Clostridium cluster XIVa (Clostridium coccoides subgroup)
ctttgagtttcattcttgcgaa

SEQ ID NO: 49 - DNA, 18 bp, Artificial Sequence
  Primer, Clostridium cluster IV (Clostridium leptum)
ccttccgtgccgsagtta

SEQ ID NO: 50 - DNA, 26 bp, Artificial Sequence
  Primer, Clostridium cluster IV (Clostridium leptum)
gaattaaaccacatactccactgctt

SEQ ID NO: 51 - DNA, 18 bp, Artificial Sequence
  Primer, Bacteroides
gagaggaaggtcccccac

SEQ ID NO: 52 - DNA, 19 bp, Artificial Sequence
  Primer, Bacteroides
cgctacttggctggttcag

SEQ ID NO: 53 - DNA, 20 bp, Artificial Sequence
  Primer, Bifidobacterium
cgggtgagtaatgcgtgacc

SEQ ID NO: 54 - DNA, 18 bp, Artificial Sequence
  Primer, Bifidobacterium
tgataggacgcgacccca

SEQ ID NO: 55 - DNA, 50 bp, Artificial Sequence
  Modified primer 8F
  misc_feature (30)..(31): barcode
ccatctcatccctgcgtgtctccgactcagagrgtttgatymtggctcag

SEQ ID NO: 56 - DNA, 49 bp, Artificial Sequence
  Modified Primer 338R
cctatcccctgtgtgccttggcagtctcagtgctgcctcccgtaggagt

SEQ ID NO: 57 - DNA, 19 bp, Artificial Sequence
  KOD FX (TOYOBO), 16S rRNA gene-specific primer, 8F
gagtttgatcmtggctcag

SEQ ID NO: 58 - DNA, 16 bp, Artificial Sequence
  KOD FX (TOYOBO), 16S rRNA gene-specific primer, 519R
attaccgcggckgctg

SEQ ID NO: 59 - DNA, 21 bp, Artificial Sequence
  KOD FX (TOYOBO), 16S rRNA gene-specific primer, 1513R
acggctaccttgttacgactt

SEQ ID NO: 60 - DNA, 20 bp, Artificial Sequence
  16S rRNA gene-specific primer
agagtttgatcmtggctcag

SEQ ID NO: 61 - DNA, 16 bp, Artificial Sequence
  16S rRNA gene-specific
attaccgcggckgctg

SEQ ID NO: 62 - DNA, 17 bp, Artificial Sequence
  Primer, total bacteria
ggtgaatacgttcccgg

SEQ ID NO: 63 - DNA, 22 bp, Artificial Sequence
  Primer, total bacteria
tacggctaccttgttacgactt

SEQ ID NO: 64 - DNA, 20 bp, Artificial Sequence
  Primer, Clostridium cluster XIVa (Clostridium coccoides subgroup)
aaatgacggtacctgactaa

SEQ ID NO: 65 - DNA, 22 bp, Artificial Sequence
  Clostridium cluster XIVa (Clostridium coccoides subgroup)
ctttgagtttcattcttgcgaa

SEQ ID NO: 66 - DNA, 16 bp, Artificial Sequence
  Primer, Clostridium cluster IV (Clostridium leptum)
gcacaagcagtggagt

SEQ ID NO: 67 - DNA, 18 bp, Artificial Sequence
  Primer, Bacteroides
gagaggaaggtcccccac

SEQ ID NO: 68 - DNA, 19 bp, Artificial Sequence
  Primer, Bacteroides
cgctacttggctggttcag

SEQ ID NO: 69 - DNA, 18 bp, Artificial Sequence
  Primer, Clostridium cluster IV (Clostridium leptum)
cttcctccgttttgtcaa

SEQ ID NO: 70 - DNA, 323 bp, Artificial Sequence
  OTU3
gatgaacgctggcggcgtgcttaacacatgcaagtcgagcgaagcactaagacggatttcttcggattgaagtctttgtgactgagcggcggacggtgagtaacgcgtgggtaacctgcctcatacagggggataacagttagaaatgactgctaataccgcataagcgcacaggaccgcatggtctggtgtgaaaaactccggtggtatgagatggacccgcgtctgattagctagttggagggtaacggcccaccgaaggcgacgatcagtagccggcctgagagggtgaacggccacattgggactgagacacggcccag

SEQ ID NO: 71 - DNA, 324 bp, Artificial Sequence
  OTU15
gatgaacgctggcggcgtgcttaacacatgcaagtcgagcgaagcattaagacagatttcttcggattgaagtctttgtgactgagcggcggacgggtgagtaacgcgtgggtaacctgcctcatacagggggataacagttagaaatgactgctaataccgcataagcgcacagggccgcatggtctggtgtgaaaaactccggtggtgtaagatggacccgcgtctgattaggtagttggtggggtaacggcccaccaagccgacgatcagtagccgacctgagagggtgaccggccacattgggactgagacacggcccaa

SEQ ID NO: 72 - DNA, 324 bp, Artificial Sequence
  OTU23
gatgaacgctggcggcgtgcttaacacatgcaagtcgaacgaagcattttggaaggaagttttcggatggaattccttaatgactgagtggcggacgggtgagtaacgcgtggggaacctccctactacaggggagtaacagctggaacggactgctaataccgcataagcgcacagaatcgcatgattcggtgtgaaagctccggcagtataggatggtcccgcgtctgattagctggttggcgggtaacggcccaccaaggcgacgatcagtagccggcttgagagagtggacggccacattgggactgagacacggcccaa

SEQ ID NO: 73 - DNA, 324 bp, Artificial Sequence
  OTU38
gatgaacgctggcggcgtgcttaacacatgcaagtcgagcgaagcggtttcaatgaagttttcggatggaattgaaattgacttagcggcggacgggtgagtaacgcgtgggtaacctgcctcatacagggggataacagttagaaatgactgctaataccgcataagcgcacaggaccgcatggtctggtgtgaaaaactccggtggtatgagatggacccgcgtctgattagctagttggaggggtaacggcccaccaaggcgacgatcagtagccggcctgagagggtgaacggccacattgggactgagacacggcccag

SEQ ID NO: 74 - DNA, 328 bp, Artificial Sequence
  OTU49
gatgaacgctggcggcgtgcctaacacacgcaagacgaacgaagcaattaaaatgaagttttcggatggatttttgattgactgagtggcggacgggtgagtaacgcgtggataacctgcctcacactggggggataacagttagaaatgactgctaataccgcataagcgcacagtaccgcatggtacgtgtgaaaactaccggtggtgtgagatggagtcccgcgtctgattagccagttggcggggtaacggcccaccaaagcgacgatcagtagccgacctgagagggtgaccggccacattggggactgagacacgggcccaa

SEQ ID NO: 75 - DNA, 324 bp, Artificial Sequence
  OTU57
gatgaacgctggcggcgtgcttaacacatgcaagtcgagcgaagcggtttcgatgaagttttcggatggatttgaaatcgacttagcggcggacgggtgagtaacgcgtgggtaacctgccttacactgggggataacagttagaaatgactgctaataccgcataagcgcacagggccgcatggtctggtgcgaaaaactccggtggtgtaagatggacccgcgtctgattagccagttggcagggtaacggcctaccaaagcgacgatcagtagccggcctgagagggtgaacggccacattgggactgagacacggcccaa

SEQ ID NO: 76 - DNA, 327 bp, Artificial Sequence
  OTU89
gatgaacgctggcggcgtgcttaacacatgcaagtcgaacgaagcattttggaaggaagttttcggatggaatcggtataacttagtggcggacgggtgagtaacgcgtgggaaacctgccctgtaccgggggataacacttagaaataggtgctaacaccgcataagcgcacggaaccgcatggttctgtgtgaaaaaactccggtggtacaggatggtcccgcgtctgattagccagttggcgagggtaacggcctaccaaagacgacgatcagtagccggcctgagagggtgaacggccacattgggactgagacacggcccaa

SEQ ID NO: 77 - DNA, 322 bp, Artificial Sequence
  OTU92
gatgaacgctggcggcgtgcctaacacatgcaagtcgaacggagttatgcagaggaagttttcggatggaatcggcgtaacttagtggcggacgggtgagtaacgcgtgggaaacctgccctgtaccgggggataacacttagaaataggtgctaataccgcataagcgcacagcttcacatgaggcagtgtgaaaaactccggtggtgtaagatggacccgcgtctgattaggtagttggtggggtaacggcccaccaagccgacgatcagtagccgacctgagagggtgaccggccacattgggactgagacacggccca

SEQ ID NO: 78 - DNA, 323 bp, Artificial Sequence
  OTU101
gatgaacgctggcggcgtgcctaacacatgcaagtcgaacgaagcaattaagatgaagttttcggatggaatcttgattgactgagtggcggacgggtgagtaacgcgtggataacctgcctcacactgggggataacagttagaaatgactgctaataccgcataagcgcacagtgccgcatggcagtgtgtgaaaaactccggtggtgtgagatggatccgcgtctgattagccagttggcggggtaacggccaccgaaagcgacgatcagtagccgacctgagagggtgaccggccacactgggactgagacacggccca

SEQ ID NO: 79 - DNA, 322 bp, Artificial Sequence
  OTU111
gatgaacgctggcggcgtgcctaacacatgcaagtcgaacgaagttacacagaggaagttttcggatggaatcggtataacttagtggcggacgggtgagtaacgcgtgggaaacctgccctgtaccgggggataacacttagaaataggtgctaataccgcataagcgcacagcttcacatgaagcagtgtgaaaaactccggtggtacaggatggtcccgcgtctgattagctggttggcggggtaacggcccaccaaggcgacgatcagtagccggcttgagagagtggacggccacattgggactgagacacggccca

SEQ ID NO: 80 - DNA, 323 bp, Artificial Sequence
  OTU114
gatgaacgctggcggcgtgcctaacacatgcaagtcgagcgaagcgctgttttcagaatcttcggaggaagaggacagtgactgagcggcggacgggtgagtaacgcgtgggcaacctgcctcatacagggggataacagttagaaatgactgctaataccgcataagcgcacaggaccgcatggtgtagtgtgaaaaactccggtggtatgagatggacccgcgtctgattagccagttggcagggtaacggcctaccaaagcgacgatcagtagccggcctgagagggtgaacggccacattgggactgagacacggccca

SEQ ID NO: 81 - DNA, 324 bp, Artificial Sequence
  OTU119
  misc_feature (293)..(293): n is a, c, g, or t
gatgaacgctggcggcgtgcctaacacatgcaagtcgaacgaagcaattaagatgaagttttcggatggaatcttgattgactgagtggcggacgggtgagtaacgcgtggataacctgcctcacactgggggataacagttagaaatgactgctaataccgcataagcgcacagtgccgcatggcagtgtgtgaaaaactccggtggtgtgagatggatccgcgtctgattagccagttgcggggtaacggcccgaccaaagcgacggatcagtagccgacctgagagggtnaccggccacattgggactgagacacggccca

SEQ ID NO: 82 - DNA, 325 bp, Artificial Sequence
  OTU125
gatgaacgctggcggcgtgcctaacacatgcaagtcgagcgaagcgctgttttcagaatcttcggaggaagaggacagtgactgagcggcggacgggtgagtaacgcgtgggcaacctgcctcatacagggggataacagttagaaatgactgctaataccgcataagcgcacaggaccgcatggtgtagtgtgaaaaactccggtggtatgagatggacccgcgtctgattaggtagttggtgggtaaaggctaccgaagccgacgatcagtagccgacctgacgagggtgaccggccacgattgggactgagacacggcccaa

SEQ ID NO: 83 - DNA, 322 bp, Artificial Sequence
  OTU131
  misc_feature (291)..(291): n is a, c, g, or t
gatgaacgctggcggcgtgcctaacacatgcaagtcgaacgaagcaattaagatgaagttttcggatggaatcttgattgactgagtggcggacgggtgagtaacgcgtggataacctgcctcacactgggggataacagttagaaatgactgctaataccgcataagcgcacagtgccgcatggcagtgtgtgaaaaactccggtggtgtgagatggatccgcgtctgattagccagttgcgggtaacggccaccgaaagcgacgatcagtagccgacctgacgagggtnaccggcacattgggactgagacacggcccaa

SEQ ID NO: 84 - DNA, 325 bp, Artificial Sequence
  OTU137
gatgaacgctggcggcgtgcctaacacatgcaagtcgaacgaagcaattaagatgaagttttcggatggaatcttgattgactgagtggcggacgggtgagtaacgcgtggataacctgcctcacactggggggataacagttagaaatgactgctaataccgcataagcgcacagtgccgcatggcagtgtgtgaaaaactccggtggtgtgagatggatccgcgtctgattaggtagttggtggggtaacggcccaccaagccgacgatcagtagccgacctgagagggtgaccggccacattgggactgagacacggcccaa

SEQ ID NO: 85 - DNA, 325 bp, Artificial Sequence
  OTU144
gatgaacgctggcggcgtgcttaacacatgcaagtcgagcgaagcggtttcgatgaagtttttggatggaattgaaattgacttagcggcggacgggtgagtaacgcgtgggtaacctgccttacactgggggataacagttagaaatgactgctaataccgcataagcgcacagggccgcatggtctggtgcgaaaaactccggtggtgtaagatggacccgcgtctgattaggtagttggtggggtaacggcccaccgaagccgacgatcagtagccgacctgagagggtgaccggcacattgggacctgagacacgggccca

SEQ ID NO: 86 - DNA, 324 bp, Artificial Sequence
  OTU161
gatgaacgctggcggcgtgcctaacacatgcaagtcgaacgaagcattttagatgaagttttcggatggattctgagatgactgagtggcggacgggtgagtaacacgtggataacctgcctcacactgggggacaacagttagaaatgactgctaataccgcataagcgcacagtaccgcatggtacggtgtgaaaaactccggtggtacaggatggtcccgcgtctgattagccagttggcagggtaacggcctaccaaagcgacgatcagtagccggcctgagagggtgaacggccacattgggactgagacacggcccaa

SEQ ID NO: 87 - DNA, 322 bp, Artificial Sequence
  OTU163
gatgaacgctggcggcgtgcctaacacatgcaagtcgaacgaagttacacggaggaagttttcggatggaatcggtataacttagtggcggacgggtgagtaacgcgtgggaaacctgccctgtaccgggggataacacttagaaataggtgctaataccgcataagcgcacggaaccgcatggttccgtgtgaaaaactccggtggtacaggatggtcccgcgtctgattaggtagttggtggggtaacggcccaccaagccgacgatcagtagccgacctgagagggtgaccggccacattgggactgagacacggccca

SEQ ID NO: 88 - DNA, 327 bp, Artificial Sequence
  OTU165
gatgaacgctggcggcgtgcttaacacatgcaagtcgaacggagcacccttgactgaggtttcggccaaatgataggaatgcttagtggcggactggtgagtaacgcgtgaggaacctaccttccagaggggacgaacagttggaacgactgctaataccgcatgacgcatgaccggggcgatcccgggccgatgtcaaagattttattcgctggaagatggcctcgcgtctgattagctagatggtggggtaacggcccaccatggcgacgatcagtagccggactgagaggttgaccggccacattgggactgagatacggccca

SEQ ID NO: 89 - DNA, 327 bp, Artificial Sequence
  OTU181
gatgaacgctggcggcgtgcctaacacatgcaagtcgaacgaagcaatttaaaatgaagttttcggatggatttttgattgactgagtggcggacgggtgagtaacgcgtggataacctgcctcacgactgggggataacagttagaaatgactgctaataccgcataagcgcacagtaccgcatggtacggtgtgaaaaactccggtggtgtgagatggatccgcgtctgattagccagttgcggggtaacggcccaccgaaagcgacgatcagtagccgacctgagagggtgaccggccacattggggactgagacacggcccaa

SEQ ID NO: 90 - DNA, 300 bp, Artificial Sequence
  OTU182
gatgaacgctggcggcgtgcctaatacatgcaagtcgaacgcgggcagcaatgcccgagtggcgaacgggtgagtaatacataagtaacctgccctttacagggggataactattggaaacgatagctaagaccgcataggtaaagataccgcatggtaagtttattaaaagtgccaaggcactacgagggagtagtgatatgcgcatagctagttggtgaggtaacggctcaccaaggcgacgatgcgtagccgacctgagagggtgaccggccacactgggactgagacacggcccag

SEQ ID NO: 91 - DNA, 323 bp, Artificial Sequence
  OTU189
gatgaacgctggcggcgtgcctaacacatgcaagtcgaacgaagcattttagatgaagttttcggatggattctgagatgactgagtggcggacgggtgagtaacacgtggataacctgcctcacactgggggacacagttagaaatgactgctaataccgcataagcgcacagcttcacatgaagcagtgtgaaaaactccggtggtacaggatggtcccgcgtctgattagccagttggcagggtaacggcctaccaaagcgacgatcagtagccggcctgagagggtgaacggccacattgggactgagacacggcccag

SEQ ID NO: 92 - DNA, 322 bp, Artificial Sequence
  OTU196
gacgaacgctggcggcgtgcttaacacatgcaagtcgaacggagcacccctgaatgaggtttcggccaaaggaagggaatgcttagtggcggactggtgagtaacgcgtgaggaacctgcctttcagaggggacaacagttggaaacgactgctaataccgcatgacacatgaatggggcatcccattgatgtcaaagatttatcgctgaaagatggcctcgcgtcccattagctagtaggcggggtaacggcccacctaggcgacgatgggtagccggactgagaggttgaccggccacattgggactgagatacggccca

SEQ ID NO: 93 - DNA, 307 bp, Artificial Sequence
  OTU199
gatgaacgctggcggcgtgcctaatacatgcaagtcgaacgcgagcacttgtgctcgagtggcgaacgggtgagtaatacataagtaacctgccctagacagggggagtaactattggaacgatagctaagaccgcataggtacggacactgcgtggtgaccgtattaaaagtagcctcaaagacactggtagaggatggacttatggcgcattagctggttggcggggtaacggcccacccaaggcgacgatgcgtagccgacctgagagggtgaccggccacactgggactgagacacggcccag

SEQ ID NO: 94 - DNA, 324 bp, Artificial Sequence
  OTU202
gatgaacgctggcggcgtgcctaacacatgcaagtcgaacgaagcaatttaacggaagttttcggatggaagttgaattgactgagtggcggacgggtgagtaacgcgtgggtaacctgccttgtactgggggacaacagttagaaatgactgctaataccgcataagcgcacagtatcgcatgatacagtgtgaaaaactccggtggtacaagatggacccgcgtctgattagctagttggaggggtaacggcccaccaaggcgacgatcagtagccggcctgagagggtgaacggccacattgggactgagacacggcccag

SEQ ID NO: 95 - DNA, 323 bp, Artificial Sequence
  OTU204
gatgaacgctggcggcgtgcttaacacatgcaagtcgagcgaagcactaagacggatttcttcggattgaagtctttgtgactgagcggcggacgggtgagtaacgcgtgggtaacctgcctcatacagggggataacagttagaaatgactgctaataccgcataagaccacagtaccgcatggtacagtgggaaaaactccggtggtatgagatggacccgcgtctgattagctagttggtaaggtaacggcttaccaaggcgacgatcagtagccgacctgagagggtgaccggccacattgggactgagacacggccca

SEQ ID NO: 96 - DNA, 324 bp, Artificial Sequence
  OTU211
gatgaacgctggcggcgtgcttaacacatgcaagtcgagcgaagcggtttcgatgaagttttcggatggatttgaaatcgacttagcggcggacgggtgagtaacgcgtgggtaacctgccttacactgggggataacagctggaaacggctgctaataccgcataagcgcacagaatcgcatgattcggtgcgaaaagctccggcagtataggatggtcccgcgtctgattagctggttggcggggtaacggcccaccaaggcgacgatcagtagccggcttgagagagtggacggccacattgggactgagacacggcccaa

SEQ ID NO: 97 - DNA, 324 bp, Artificial Sequence
  OTU214
gatgaacgctggcggcgtgcctaacacatgcaagtcgaacgaagcaattaagatgaagttttcggatggaatcttgattgactgagtggcggacgggtgagtaacgcgtgggtaacctgcctcatacagggggagtaacagttagaaatgactgctaataccgcataagcgcacagggctgcatggcctggtgtgaaaaactccggtggtatgagatggacccgcgtctgattagctagttggaggggtaacggcccaccaaggcgacgatcagtagccggcctgagagggtgaacggccacattgggactgagacacggccca

SEQ ID NO: 98 - DNA, 323 bp, Artificial Sequence
  OTU224
gatgaacgctggcggcgtgcttaacacatgcaagtcgagcgaagcaccttggcggatttcttcggattgaagccttggtgactgagcggcggacgggtgagtaacgcgtgggtaacctgccctgtaccgggggataacacttagaaataggtgctaataccgcataagcgcacagcttcacatgaagcagtgtgaaaaactccggcggtacaggatggtcccgcgtctgattagccagttgacagggtaacggcctaccaaagcgacgatcagtagccggcctgagagggtgaacggccacattgggactgagacacggccca

SEQ ID NO: 99 - DNA, 324 bp, Artificial Sequence
  OTU225
gatgaacgctggcggcgtgcctaacacatgcaagtcgaacggaagttatgcagaggaagttttcggtatggaatcggcgtaacttagtggcggacgggtgagtaacgcgtgggaaacctgccctgtaccgggggagtaacacttagaataggtgctaataccgcataagcgcacagcttcacatgaggcagtgtgaaaaactccggtggtacaggatggtcccgcgtctgattagccagttggcagggtaacggcctaccaaagcgacgatcagtagccggcctgagagggtgaacggccacattgggactgagacacggccca

SEQ ID NO: 100 - DNA, 322 bp, Artificial Sequence
  OTU237
gatgaacgctggcggcgtgcctaacacatgcaagtcgaacgaagcaattgaaggaagttttcggatggaattcgattgactgagtggcggacgggtgagtaacgcgtggataacctgcctcacactgggggataacagttagaaatgactgctaataccgcataagcgcacagtgccgcatggtacggtgtgaaaaactccggtggtgtgagatggatccgcgtctgattagccagttggcggggtaacggcccaccaaagcgacgatcagtagccgacctgagagggtgaccggccacattgggactgagacacggcccaa

SEQ ID NO: 101 - DNA, 323 bp, Artificial Sequence
  OTU246
gatgaacgctggcggcgtgcctaacacatgcaagtcgaacggagttatgcagaggaagttttcggatggaatcggcgtaacttagtggcggacgggtgagtaacgcgtgggaaacctgccctatacagggggataacagctggaaacggctgctaataccgcataagcgcacagaatcgcatgattcggtgtgaaaagctccggcagtataggatggtcccgcgtctgattagctggttggcggggtaacggcccaccaaggcgacgatcagtagccggcttgagagagtggacggccacattgggactgagacacggcccaa

SEQ ID NO: 102 - DNA, 325 bp, Artificial Sequence
  OTU262
gatgaacgctggcggcgtgcctaacacatgcaagtcgaacgaagcattttagatgaagttttcggatggattctgagatgactgagtggcggacgggtgagtaacacgtggataacctgcctcacactgggggacaacagttagaaatgactgctaataccgcataagcgcacagtaccgcatggtacagtgtgaaaaactccggtggtgtgagatggatccgcgtctgattagccagttggcggggtaacggcccaccaaagcgacgatcagtagccgacctgagagggtgaccggccacattggggacctgagacacggccca

SEQ ID NO: 103 - DNA, 326 bp, Artificial Sequence
  OTU268
gatgaacgctggcggcgtgcctaacacatgcaagtcgagcgaagcgctgttttcagaatcttcggaggaagaggacagtgactgagcggcggacgggtgagtaacgcgtgggcaacctgcctcatacagggggataacagttagaaatgactgctaataccgcataagcgcacaggaccgcatggtgtagtgtgaaaaactccggtggtatgagatggacccgcgtctgattaggtagttggtggggtaaaggcctaccaagccgacgatcagtagccgacctgagacgggtgaccggcacattggggactgagacacgggcccaa

SEQ ID NO: 104 - DNA, 329 bp, Artificial Sequence
  OTU269
gatgaacgctggcggcgtgcctaacacatgcaagtcgaacgaagcattttagatgaagttttcggatggattctgagatgactgagtggcggacgggtgagtaacacgtggataacctgcctcacactgggggacgaacagttagaaatagactgctaataccgcataagcgcacagtaccgcatggtacagtgtgaaaaactaccggtggtgtgagatggatccgcgctgattagtccagttggcggggtaacggccgaccaaagcgacgatcagtagccgacctgagagggtgaccggccgacagttgggactgagacacggcccaa

SEQ ID NO: 105 - DNA, 326 bp, Artificial Sequence
  OTU277
gatgaacgctggcggcgtgcttaacacatgcaagtcgagcgaagcactaagacggatttctttggattgaagtctttgtgactgagcggcggacgggtgagtaacgcgtgggtaacctgcctcatacagggggataacagttagaaatgactgctaataccgcataagcgcacaggatcgcatggtctggtgtggaaaaactccggtggtatgagatggacccgcgtctgattagctagttggaggggtaacggcccaccaaggcgacgatcagtagccggcctgagagggtgaacggccacgattgggactgagacacggcccag

SEQ ID NO: 106 - DNA, 323 bp, Artificial Sequence
  OTU279
gatgaacgctggcggcgtgcctaacacatgcaagtcgaacgaagttagacagaggaagttttcggatggaatcggtataacttagtggcggacgggtgagtaacgcgtgggaacctgccctgtaccgggggagtaacacttagaaataggtgctaataccgcataagcgcacggaaccgcatggttctgtgtgaaaaactaccggtggtacaggatggtcccgcgtctgattagccagttggcagggtaacggcctaccaaagcgacgatcagtagccggcctgagagggtgaacggccacattgggactgagacacggccca

SEQ ID NO: 107 - DNA, 315 bp, Artificial Sequence
  OTU280
gatgaacgctggcggcgtgcctaatacatgcaagtcgaacgctttgtaaaggagcttgcttctttacgaggagtggcgaacgggtgagtaatacataagcaatctgcccatcggcctgggataacagttggaaacgactgctaataccggataggttagtttctggcatcagggactaattaaagttgggatacaacacggatggatgagcttatggcgtattagctagtaggtgaggtaacggcccacctaggcgatgatacgtagccgacctgagagggtgaccggccacattgggactgagacacggcccaa

SEQ ID NO: 108 - DNA, 325 bp, Artificial Sequence
  OTU286
gatgaacgctggcggcgtgcttaacacatgcaagtcgagcgaagcactaagacggatttcttcggattgaagtctttgtgactgagcggcggacgggtgagtaacgcgtgggtaacctgcctcatacagggggataacagttagaaatgactgctaataccgcataagcgcacaggatcgcatggtctggtgtgaaaaactccggtggtatgagatggacccgcgtctgattagccagttggcagggtaacggcctaccaaagcgacgatcagtagccggcctgagagggtgaacggccacattgggactgagacacgggcccaa

SEQ ID NO: 109 - DNA, 329 bp, Artificial Sequence
  OTU287
gacgaacgctggcggcgcgcctaacacatgcaagtcgaacggacacatccgacggaatagcttgctaggaagatggatgttgttagtggcggacgggtgagtaacacgtgagcaacctgcctcggagtgggggacaacagttggaaacgactgctaataccgcatacggtggtcgggggacatcccctggccaagaaaggattatatccgctctgagatgggctcgcgtctgattagctagttggcgggtaatggcccgaccgaaggcaacgatcagtagccggactgagaggttgaacggccacattgggactgagacacggccccag

SEQ ID NO: 110 - DNA, 328 bp, Artificial Sequence
  OTU297
gatgaacgctggcggcgtgcctaacacatgcaagtcgaacgaagcatcttataggaagttttcggatggaatatgggatgactgagtggcggacgggtgagtaacgcgtggataacctgcctcacactgggggagtaacagttagaaatggctgctaataccccactaagcgcacggtaccgcatggtacggtgtgaaaaacccaggtggtgtgagatggatccgcgtctgattagccagttggcggggtaacggcccgaccaaacgcgacgatcagtagccgacctgagagggtgaccggccgacattgggactgagacacggccca

SEQ ID NO: 111 - DNA, 326 bp, Artificial Sequence
  OTU303
gatgaacgctggcggcgtgcctaacacatgcaagtcgaacgaagcattttagatgaagttttcggatggattctgagatgactgagtggcggacgggtgagtaacacgtggataacctgcctcacactgggggacaacagttagaaatgactgctaataccgcataagcgcacagtaccgcatggtacagcgtgaaaaactccggtggtgtgagatggatccgcgtctgattagccagttggcggggtaacggcccaccaaagcgacgatcagtagccgacctgagagggtgaccggcacattggggactgagaccacgggcccaa

SEQ ID NO: 112 - DNA, 310 bp, Artificial Sequence
  OTU304
attgaacgctggcggcaggcctaacacatgcaagtcgaacggtaacaggaagcagcttgctgctttgctgacgagtggcggacgggtgagtaatgtctgggaaactgcccgatggagggggataactactggaaacggtagctaataccgcataacgtcgcaagaccaaagagggggaccttagggcctcttgccatcggatgtgcccagatgggattagctagtaggtggggtaaaggctcacctaggcgacgatccctagctggtctgagaggatgaccagccacactggaactgagacacggtccag

SEQ ID NO: 113 - DNA, 325 bp, Artificial Sequence
  OTU307
gatgaacgctggcggcgtgcctaacacatgcaagtcgaacgaagcatcttataggaagttttcggatggaatatgggatgactgagtggcggacgggtgagtaacgcgtggagtaacctgcctcacactgggggataacagttagaaatggctgctaataccccataagcgcacagtaccgcatggtacggtgtgaaaaacccaggtggtgtgagatggatccgcgtctgattagccagttggcgggtaacggccgaccaaagcgacgatcagtagccgacctgagagggtgaccggcacgattgggacctgagacacgggccca

SEQ ID NO: 114 - DNA, 323 bp, Artificial Sequence
  OTU312
gatgaacgctggcggcgtgcctaacacatgcaagtcgaacgaagttatatcgaggaagttttcggatggaatcagtataacttagtggcggacgggtgagtaacgcgtgggaaacctgccctgtaccgggggataacacttagaaataggtgctaataccgcataagcgcacagcttcacatgaagcagtgtgaaaaactccggtggtatgagatggacccgcgtctgattagctagttggaggggtaacggcccaccaaggcgacgatcagtagccggcctgagagggtgaacggccacattgggactgagacacggcccag

SEQ ID NO: 115 - DNA, 301 bp, Artificial Sequence
  OTU313
gatgaacgctggcggcgtgcctaatacatgcaagtcgaacgcgggcagcaatgcccgagtggcgaacgggtgagtaatacataagtaacctgccctttacagggggataactattggaaacgatagctaagaccgcataggtaaagataccgcatggtaagtttattaaagtgccaaggcactggtagaggatggacttatggcgcattagctagttggtgaggtaacggctcaccaaggcgacgatgcgtagccgacctgagagggtgaccggccacactgggactgagacacggcccaa

SEQ ID NO: 116 - DNA, 322 bp, Artificial Sequence
  OTU319
gatgaacgctggcggcgtgcctaacacatgcaagtcgaacgaagttagacagaggaagttttcggatggaatcggtataacttagtggcggacgggtgagtaacgcgtgggaaacctgccctgtaccgggggataacacttagaaatgactgctaataccgcataagcgcacagtaccgcatggtacagtgtgaaaaactccggtggtgtgagatggatccgcgtctgattagccagttggcggggtaacggcccaccaaagcgacgatcagtagccgacctgagagggtgaccggcacattgggactgagacacggcccaa

SEQ ID NO: 117 - DNA, 324 bp, Artificial Sequence
  OTU326
gatgaacgctggcggcgtgcctaacacatgcaagtcgaacgaagcaattaaaatgaagttttcggatggatttttgattgactgagtggcggacgggtgagtaacgcgtggataacctgcctcacactgggggataacagttagaaatgactgctaataccgcataagcgcacagcttcacatgaagcagtgtgaaaaactccggtggtacaggatggtcccgcgtctgattagccagttggcagggtaacggcctaccaaagcgacgatcagtagccggcctgagagggtgaacggccacattgggactgagacacggcccaa

SEQ ID NO: 118 - DNA, 324 bp, Artificial Sequence
  OTU328
gatgaacgctggcggcgtgcttaacacatgcaagtcgaacggagtgccttagaaagaggattcgtccaattgataaggttacttagtggcggacgggtgagtaacgcgtgaggaacctgcctcggagtggggaataacagaccgaaaggtctgctaataccgcatgatgcagttggaccgcatggtcctgactgccaaagatttatcgctctgagatggcctcgcgtctgattagcttgttggcggggtaatggcccaccaaggcgacgatcagtagccggactgagaggttggccggccacattgggactgagacacggccca

SEQ ID NO: 119 - DNA, 323 bp, Artificial Sequence
  OTU333
gatgaacgctggcggcgtgcttaacacatgcaagtcgaacggagtgctcatgacagaggattcgtccaatggagtgagttacttagtggcggacgggtgagtaacgcgtgagtaacctgccttggagtggggaataacaggtggaaacatctgctaataccgcatgatgcagttgggtcgcatggctctgactgccaaagatttatcgctctgagatggactcgcgtctgattagctggttggcgggtaacggccaccaaggcgacgatcagtagccggactgagaggttggccggccacattgggactgagacacggcccag

SEQ ID NO: 120 - DNA, 323 bp, Artificial Sequence
  OTU339
gatgaacgctggcggcgtgcctaacacatgcaagtcgaacgaagcaattaaaatgaagttttcggatggatttttgattgactgagtggcggacgggtgagtaacgcgtggataacctgcctcacactggggataacagttagaaatgactgctaataccgcataagcgcacagtaccgcatggtacggtgtgaaaaactccggtggtgtgagatggatccgcgtctgattagccagttgcggggtaacggcccgaccaagcgacgatcagtagccgaccgtgagaggtgaccggcccacattgggactgagacacggcccaa

SEQ ID NO: 121 - DNA, 315 bp, Artificial Sequence
  OTU340
gacgaacgctggcggcgcgcctaacacatgcaagtcgaacggagttgtgttgaaagcttgctggatatacaacttagtggcggacgggtgagtaacacgtgagtaacctgcctctcagagtggaataacgtttggaaacgaacgctaataccgcataacgtgagaagagggcatcctctttttaccaaagatttatcgctgagagatgggctcgcggccgattaggtagttggtgagataacagcccaccaagccgacgatcggtagccggactgagaggttgatcggccacattgggactgagacacggcccag

SEQ ID NO: 122 - DNA, 325 bp, Artificial Sequence
  OTU353
gatgaacgctggcggcgtgcttaacacatgcaagtcgagcgaagcaccttgacggattcttcggattgaagccttggtgactgagcggcggacgggtgagtaacgcgtgggtaacctgcctcatacaggggggataaacagttagaaatgactgctaataccgcataagcgcacaggaccgcatggtctggtgtgaaaaactccggtggtatgagatggacccgcgtctgattagctagttggaggggtaacggcccaccaaggcgacgatcagtagccggcctgagagggtgaacggccacattgggactgaggacacggccca

SEQ ID NO: 123 - DNA, 317 bp, Artificial Sequence
  OTU173
gacgaacgctggcggcgcgcctaacacatgcaagtcgaacggagttgtgttgaaagcttgctggatatacaacttagtggcggacgggtgagtaacgcgtgggtaacctgcctcatacagggggataacagttagaaatgactgctaataccgcataagcgcacaggatcgcatggtctggtgtgaaaaactccggtggtatgagatggacccgcgtctgattaactagttggaggggtaacggcccaccaaggcgacgagtcagtagccggcctgagagggtgaacggccacgattgggactgagacacggcccag